European Patent Application EP 4 389 898 A2, published June 26, 2024. Title: T CELL RECEPTORS. Applicant: ADAPTIMMUNE LIMITED. Application EP 24170484.0, filed April 10, 2017. The sequence listing filed with the application follows.

SEQUENCE LISTING (29 sequences)

SEQ ID NO: 1 - protein, 10 aa, Homo sapiens
GVYDGEEHSV

SEQ ID NO: 2 - protein, 10 aa, Homo sapiens
GVYDGREHTV

SEQ ID NO: 3 - protein, 105 aa, synthetic construct
MKNQVEQSPQSLIILEGKNCTLQCNYTVSPFSNLRWYKQDTGRGPVSLTIMTFSENTKSNGRYTATLDADTKQSSLHITASQLSDSASYICVVSGGTDSWGKLQF

SEQ ID NO: 4 - protein, 123 aa, synthetic construct
MASLLFFCGAFYLLGTGSMDADVTQTPRNRITKTGKRIMLECSQTKGHDRMYWYRQDPGLGLRLIYYSFDVKDINKGEISDGYSVSRQAQAKFSLSLESAIPNQTALYFCATSGQGAYNEQFF

SEQ ID NO: 5 - protein, 229 aa, synthetic construct
MKKHLTTFLVILWLYFYRGNGKNQVEQSPQSLIILEGKNCTLQCNYTVSPFSNLRWYKQDTGRGPVSLTIMTFSENTKSNGRYTATLDADTKQSSLHITASQLSDSASYICVVSGGTDSWGKLQFGAGTQVVVTPDIQNPDPAVYQLRDSKSSDKSVCLFTDFDSQTNVSQSKDSDVYITDKTVLDMRSMDFKSNSAVAWSNKSDFACANAFNNSIIPEDTFFPSPESS

SEQ ID NO: 6 - protein, 262 aa, synthetic construct
MASLLFFCGAFYLLGTGSMDADVTQTPRNRITKTGKRIMLECSQTKGHDRMYWYRQDPGLGLRLIYYSFDVKDINKGEISDGYSVSRQAQAKFSLSLESAIPNQTALYFCATSGQGAYNEQFFGPGTRLTVLEDLKNVFPPEVAVFEPSEAEISHTQKATLVCLATGFYPDHVELSWWVNGKEVHSGVSTDPQPLKEQPALNDSRYCLSSRLRVSATFWQNPRNHFRCQVQFYGLSENDEWTQDRAKPVTQIVSAEAWGRAD

SEQ ID NO: 7 - protein, 105 aa, synthetic construct
MKNQVEQSPQSLIILEGKNCTLQCNYTVSPFSNLRWYKQDTGRGPVSLTRMTFSENTKSNGRYTATLDADTKQSSLHITASQLSDSASYICVVSGGTDSWGKLQF

SEQ ID NO: 8 - protein, 123 aa, synthetic construct
MASLLFFCGAFYLLGTGSMDADVTQTPRNRITKTGKRIMLECSQTKGRDRMYWYRQDPGLGLRLIYYSFDVKDINKGEISDGYSVSRQAQAKFSLSLESAIPNQTALYFCATSGQGAYNEQFF

SEQ ID NO: 9 - protein, 123 aa, synthetic construct
MASLLFFCGAFYLLGTGSMDADVTQTPRNRITKTGKRIMLECSQTKGHDRMYWYRQDPGLGLRLIYYSFDVKDINKGEISDGYSVSRQAQAKFSLSLESAIPNQTALYFCATSGQGAYREQFF

SEQ ID NO: 10 - protein, 123 aa, synthetic construct
MASLLFFCGAFYLLGTGSMDADVTQTPRNRITKTGKRIMLECSQTKGHDRMYWYRQDPGLGLRLIYYSFDVKDINKGEISDGYSVSRQAQAKFSLSLESAIPNQTALYFCATSGQGAYKEQFF

SEQ ID NO: 11 - protein, 271 aa, synthetic construct
METLLGLLILWLQLQWVSSKQEVTQIPAALSVPEGENLVLNCSFTDSAIYNLQWFRQDPGKGLTSLLLIQSSQREQTSGRLNASLDKSSGRSTLYIAASQPGDSATYLCAVGGYSTLTFGKGTVLLVSPDNIQNPDPAVYQLRDSKSSDKSVCLFTDFDSQTNVSQSKDSDVYITDKTVLDMRSMDFKSNSAVAWSNKSDFACANAFNNSIIPEDTFFPSPESSCDVKLVEKSFETDTNLNFQNLSVIGFRILLLKVAGFNLLMTLRLWSS

SEQ ID NO: 12 - protein, 308 aa, synthetic construct
MSISLLCCAAFPLLWAGPVNAGVTQTPKFRILKIGQSMTLQCAQDMNHNYMYWYRQDPGMGLKLIYYSVGAGITDKGEVPNGYNVSRSTTEDFPLRLELAAPSQTSVYFCASSYSRWSPLHFGNGTRLTVTEDLNKVFPPEVAVFEPSEAEISHTQKATLVCLATGFFPDHVELSWWVNGKEVHSGVSTDPQPLKEQPALNDSRYCLSSRLRVSATFWQNPRNHFRCQVQFYGLSENDEWTQDRAKPVTQIVSAEAWGRADCGFTSVSYQQGVLSATILYEILLGKATLYAVLVSALVLMAMVKRKDF

SEQ ID NO: 13 - protein, 208 aa, synthetic construct
MQKEVEQNSGPLSVPEGAIASLNCTYSDRGSQSFFWYRQYSGKSPELIMFIYSNGDKEDGRFTAQLNKASQYVSLLIRDSQPSDSATYLCAVKMANQAGTALIFGKGTTLSVSSNIQNPDPAVYQLRDSKSSDKSVCLFTDFDSQTNVSQSKDSDVYITDKCVLDMRSMDFKSNSAVAWSNKSDFACANAFNNSIIPEDTFFPSPESS

SEQ ID NO: 14 - protein, 244 aa, synthetic construct
MQDGGITQSPKFQVLRTGQSMTLLCAQDMNHEYMYWYRQDPGMGLRLIHYSVGAGITDQGEVPNGYNVSRLNKREFSLRLESAAPSQTSVYFCASLGGLADEQFFGPGTRLTVLEDLKNVFPPEVAVFEPSEAEISHTQKATLVCLATGFYPDHVELSWWVNGKEVHSGVCTDPQPLKEQPALNDSRYALSSRLRVSATFWQDPRNHFRCQVQFYGLSENDEWTQDRAKPVTQIVSAEAWGRAD

SEQ ID NO: 15 - protein, 275 aa, synthetic construct
MKTFAGFSFLFLWLQLDCMSRGEDVEQSLFLSVREGDSSVINCTYTDSSSTYLYWYKQEPGAGLQLLTYIFSNMDMKQDQRLTVLLNKKDKHLSLRIADTQTGDSAIYFCAERNSGAGSYQLTFGKGTKLSVIPNIQNPDPAVYQLRDSKSSDKSVCLFTDFDSQTNVSQSKDSDVYITDKTVLDMRSMDFKSNSAVAWSNKSDFACANAFNNSIIPEDTFFPSPESSCDVKLVEKSFETDTNLNFQNLSVIGFRILLLKVAGFNLLMTLRLWSS

SEQ ID NO: 16 - protein, 311 aa, synthetic construct
MGTSLLCWMALCLLGADHADTGVSQNPRHKITKRGQNVTFRCDPISEHNRLYWYRQTLGQGPEFLTYFQNEAQLEKSRLLSDRFSAERPKGSFSTLEIQRTEQGDSAMYLCASSLFSGVNTEAFFGQGTRLTVVEDLNKVFPPEVAVFEPSEAEISHTQKATLVCLATGFFPDHVELSWWVNGKEVHSGVSTDPQPLKEQPALNDSRYCLSSRLRVSATFWQNPRNHFRCQVQFYGLSENDEWTQDRAKPVTQIVSAEAWGRADCGFTSVSYQQGVLSATILYEILLGKATLYAVLVSALVLMAMVKRKDF

SEQ ID NO: 17 - protein, 10 aa, Homo sapiens
GVVDGREHTV

SEQ ID NO: 18 - protein, 6 aa, synthetic construct
VSPFSN

SEQ ID NO: 19 - protein, 6 aa, synthetic construct
LTIMTF

SEQ ID NO: 20 - protein, 6 aa, synthetic construct
LTRMTF

SEQ ID NO: 21 - protein, 15 aa, synthetic construct
CVVSGGTDSWGKLQF

SEQ ID NO: 22 - protein, 5 aa, synthetic construct
KGHDR

SEQ ID NO: 23 - protein, 5 aa, synthetic construct
KGRDR

SEQ ID NO: 24 - protein, 5 aa, synthetic construct
SVFDK

SEQ ID NO: 25 - protein, 14 aa, synthetic construct
CATSGQGAYNEQFF

SEQ ID NO: 26 - protein, 14 aa, synthetic construct
CATSGQGAYREQFF

SEQ ID NO: 27 - protein, 14 aa, synthetic construct
CATSGQGAYKEQFF

SEQ ID NO: 28 - protein, 5 aa, synthetic construct
SFDVK

SEQ ID NO: 29 - protein, 123 aa, synthetic construct
MASLLFFCGAFYLLGTGSMDADVTQTPRNRITKTGKRIMLECSQTKGHDRMYWYRQDPGLGLRLIYYSFDVKDINKGEISDGYSVSRQAQAKFSLSLESAIPNQTALYFCATSGQGAYEEQFF